European Patent Application EP 4 159 743 A1, published April 5, 2023. Title: Methods for preparing pyridazine compounds. Applicant: ETH Zurich. The sequence listing filed with the application follows.

SEQUENCE LISTING (4 sequences)

SEQ ID NO: 1 - DNA, 1260 bp, Pleurocapsa sp.
atgactaaaaaatacagacgagttagttatgcagtttgggaaattaccttgaaatgcaatctagcttgtagtcactgtggttcgagagcagggcaggcaagaaccaaggaactatctacagaagaagcttttaatctggttcggcaactagccgatgtaggaatcaaagaggttactctaatcggtggcgaagcctttatgcgctctgattggctagaaattgccaaggctgttactgaggcagggatgatctgcggtatgactacaggtggatttggtgtcagtttggaaactgccagaaaaatgaaagaagctggaattaaaacagtttctgtatctatcgatggtggcataccagaaacccacgatcgccagcgagggaaaaaaggtgcttggcattctgcttttagaaccatgagccatctaaaagaagtcggcatctattttggctgcaatacccagataaaccgtttatctgcctctgaattcccaataatttacgaacgaataagggacgctggagcaagagcttggcagattcaattaactgtacctatgggtaatgcggcagataatgcagacatgttattgcaaccatacgaactattagatatttatcccatgttagctcgtgttgctaaacgagctaaacaggaaggtgttcgcatacaggcgggaaataatattggctattatggcccttatgaaagactgctgcgtggtagtgatgaatggacattttggcagggttgcggagcgggtttaaataccttgggtatcgaagctgatggcaaaattaaaggttgtccttctttacctacggctgcttatacgggcggtaatatccgcgatcgccctttaagagaaatagtcgaacagactgaagagcttaaatttaatctgaaggctgggactgaacagggcacagaccacatgtggggattttgtaaaacctgtgaatttgctgaactctgtcgaggtggttgttcttggacggctcatgtcttctttgatcgccgtgggaataatccctactgccatcatcgtgctttgaaacaggcacaaaaagacatcagagaaagattctatttaaaagtaaaagcaaaagggaatccttttgataatggggaatttgtcattatagaagaacctttcaacgcacctttgccagagaacgatttgcttcattttaatagcgatcacattcagtggccagaaaactggcaaaattctgaatctgcttacgctttagcaaagtaa

SEQ ID NO: 2 - protein, 419 aa, Pleurocapsa sp.
MTKKYRRVSYAVWEITLKCNLACSHCGSRAGQARTKELSTEEAFNLVRQLADVGIKEVTLIGGEAFMRSDWLEIAKAVTEAGMICGMTTGGFGVSLETARKMKEAGIKTVSVSIDGGIPETHDRQRGKKGAWHSAFRTMSHLKEVGIYFGCNTQINRLSASEFPIIYERIRDAGARAWQIQLTVPMGNAADNADMLLQPYELLDIYPMLARVAKRAKQEGVRIQAGNNIGYYGPYERLLRGSDEWTFWQGCGAGLNTLGIEADGKIKGCPSLPTAAYTGGNIRDRPLREIVEQTEELKFNLKAGTEQGTDHMWGFCKTCEFAELCRGGCSWTAHVFFDRRGNNPYCHHRALKQAQKDIRERFYLKVKAKGNPFDNGEFVIIEEPFNAPLPENDLLHFNSDHIQWPENWQNSESAYALAK

SEQ ID NO: 3 - DNA, 171 bp, Pleurocapsa sp.
tcatgtcagaaaattgctaatttcagcaatttctaaactttgttttgctttaattaatgctttgataaaagcttgcttgtcttgccaaccctgacgaggtaaaaccgagctggaatcatctgatttttgagctgctgtggctactttatttggtatttgattagagttcat

SEQ ID NO: 4 - protein, 56 aa, Pleurocapsa sp.
MNSNQIPNKVATAAQKSDDSSSVLPRQGWQDKQAFIKALIKAKQSLEIAEISNFLT